European Patent Application EP 4 335 930 A1, published March 13, 2024. Title: KIT FOR DETECTING MICROSATELLITE INSTABILITY AND METHOD THEREFOR. Applicant: Fuzhou University. Application CN. The sequence listing filed with the application follows.

SEQUENCE LISTING (24 sequences)

SEQ ID NO: 1 - DNA, 21 bp, synthetic construct
  source 1..21: mol_type = other DNA
ttatatttaaatgtatgtctc

SEQ ID NO: 2 - DNA, 19 bp, synthetic construct
  source 1..19: mol_type = other DNA
caagcagataaaagagaac

SEQ ID NO: 3 - DNA, 21 bp, synthetic construct
  source 1..21: mol_type = other DNA
acgcgagtgaccagaaagtgt

SEQ ID NO: 4 - DNA, 30 bp, synthetic construct
  source 1..30: mol_type = other DNA
tggcctttttttttttttttttttttagca

SEQ ID NO: 5 - DNA, 20 bp, synthetic construct
  source 1..20: mol_type = other DNA
gctgaattttacctcctgac

SEQ ID NO: 6 - DNA, 19 bp, synthetic construct
  source 1..19: mol_type = other DNA
aacctgggtgacagagtga

SEQ ID NO: 7 - DNA, 20 bp, synthetic construct
  source 1..20: mol_type = other DNA
aaaaactcttctcttccctg

SEQ ID NO: 8 - DNA, 31 bp, synthetic construct
  source 1..31: mol_type = other DNA
cctatttttttttttttttttttttttgtga

SEQ ID NO: 9 - DNA, 18 bp, synthetic construct
  source 1..18: mol_type = other DNA
ccaacgtctgtgagatcc

SEQ ID NO: 10 - DNA, 20 bp, synthetic construct
  source 1..20: mol_type = other DNA
actagcaatgaccaataagc

SEQ ID NO: 11 - DNA, 19 bp, synthetic construct
  source 1..19: mol_type = other DNA
ggaaaccatgcttgcaaac

SEQ ID NO: 12 - DNA, 34 bp, synthetic construct
  source 1..34: mol_type = other DNA
tggtaaaaaaaaaaaaaaaaaaaaaaaaaagcca

SEQ ID NO: 13 - DNA, 20 bp, synthetic construct
  source 1..20: mol_type = other DNA
acttaatatccctaaacaat

SEQ ID NO: 14 - DNA, 18 bp, synthetic construct
  source 1..18: mol_type = other DNA
gcctgggtgacataatga

SEQ ID NO: 15 - DNA, 24 bp, synthetic construct
  source 1..24: mol_type = other DNA
actacaggcatgaattactactgt

SEQ ID NO: 16 - DNA, 36 bp, synthetic construct
  source 1..36: mol_type = other DNA
ctccagttttttttttttttttttttttttttttga

SEQ ID NO: 17 - DNA, 21 bp, synthetic construct
  source 1..21: mol_type = other DNA
ccaagaatgtaagtgggagtg

SEQ ID NO: 18 - DNA, 24 bp, synthetic construct
  source 1..24: mol_type = other DNA
cattctgcattttaactatggctc

SEQ ID NO: 19 - DNA, 26 bp, synthetic construct
  source 1..26: mol_type = other DNA
ttctctaaagagttttgtgttttgtt

SEQ ID NO: 20 - DNA, 36 bp, synthetic construct
  source 1..36: mol_type = other DNA
ttgatttttttttttttttttttttttttgagaaca

SEQ ID NO: 21 - DNA, 31 bp, synthetic construct
  source 1..31: mol_type = other DNA
gacttcagccagtatatgaaattggatattg

SEQ ID NO: 22 - DNA, 36 bp, synthetic construct
  source 1..36: mol_type = other DNA
gtatatgtcaatgaaaacattttttaaccattcaac

SEQ ID NO: 23 - DNA, 23 bp, synthetic construct
  source 1..23: mol_type = other DNA
agcagtcagagcccttaaccttt

SEQ ID NO: 24 - DNA, 33 bp, synthetic construct
  source 1..33: mol_type = other DNA
aggtaaaaaaaaaaaaaaaaaaaaaaaaaaagg